European Patent Application EP 4 417 622 A1, published August 21, 2024. Title: ANTI-CD26 ANTIBODIES AND USE THEREOF. Applicant: ZonHon Biopharma Institute Inc. Application EP. The sequence listing filed with the application follows.

SEQUENCE LISTING (57 sequences)

SEQ ID NO: 1 - protein, 8 aa, Artificial sequence
GFNIKDTY

SEQ ID NO: 2 - protein, 8 aa, Artificial sequence
IEPMNGNT

SEQ ID NO: 3 - protein, 13 aa, Artificial sequence
SRGGWLLLYVMDY

SEQ ID NO: 4 - protein, 11 aa, Artificial sequence
KSLLHSNGNTY

SEQ ID NO: 5 - protein, 9 aa, Artificial sequence
FQQLEYPYT

SEQ ID NO: 6 - protein, 120 aa, Artificial sequence
QVQLVQSGAEVVKPGASVKISCKASGFNIKDTYIYWVRQRTGQGLEWIGRIEPMNGNTKYDPKFQGRLTMTANTSKNTAYLQLSSLTSEDTAVYYCSRGGWLLLYVMDYWGQGTTVTVSS

SEQ ID NO: 7 - protein, 112 aa, Artificial sequence
DIVMTQSASSLPVTPGEPASISCRSDKSLLHSNGNTYLYWFLQKPGQSPQVLIYRMSNLASGVPDRFSGSGSGTDFTLTISRVEAEDVGVYYCFQQLEYPYTFGQGTKLEIK

SEQ ID NO: 8 - protein, 120 aa, Artificial sequence
EVQLVQSGAELVKPGASVKLSCAASGFNIKDTYIYWVRQAPGQGLEWVGRIEPMNGNTKYDPKFQGRFTMTANTSKNTAYLQLSSLRSEDTAVYYCSRGGWLLLYVMDYWGQGTLVTVSS

SEQ ID NO: 9 - protein, 112 aa, Artificial sequence
DIVMTQSPSSLSVTPGERVSISCRSDKSLLHSNGNTYLYWFLQKPGQSPQVLIYRMSNLASGVPDRFSGSGSGTDFTLTISRVEAEDVGVYYCFQQLEYPYTFGQGTKLEIK

SEQ ID NO: 10 - protein, 119 aa, Artificial sequence
DVQLVQSGAEVKKPGASVKVSCKASGYTFTRYTMHWVRQAPGQGLEWIGYINPSRGYTNYADSVKGRFTITTDKSTSTAYMELSSLRSEDTATYYCARYYDDHYCLDYWGQGTTVTVSS

SEQ ID NO: 11 - protein, 106 aa, Artificial sequence
DIVLTQSPATLSLSPGERATLSCRASQSVSYMNWYQQKPGKAPKRWIYDTSKVASGVPARFSGSGSGTDYSLTINSLEAEDAATYYCQQWSSNPLTFGGGTKVEIK

SEQ ID NO: 12 - protein, 15 aa, Artificial sequence
GGGGSGGGGSGGGGS

SEQ ID NO: 13 - protein, 5 aa, Artificial sequence
GGGGS

SEQ ID NO: 14 - protein, 492 aa, Artificial sequence
DIVMTQSASSLPVTPGEPASISCRSDKSLLHSNGNTYLYWFLQKPGQSPQVLIYRMSNLASGVPDRFSGSGSGTDFTLTISRVEAEDVGVYYCFQQLEYPYTFGQGTKLEIKGGGGSGGGGSGGGGSQVQLVQSGAEVVKPGASVKISCKASGFNIKDTYIYWVRQRTGQGLEWIGRIEPMNGNTKYDPKFQGRLTMTANTSKNTAYLQLSSLTSEDTAVYYCSRGGWLLLYVMDYWGQGTTVTVSSGGGGSDVQLVQSGAEVKKPGASVKVSCKASGYTFTRYTMHWVRQAPGQGLEWIGYINPSRGYTNYADSVKGRFTITTDKSTSTAYMELSSLRSEDTATYYCARYYDDHYCLDYWGQGTTVTVSSGGGGSGGGGSGGGGSDIVLTQSPATLSLSPGERATLSCRASQSVSYMNWYQQKPGKAPKRWIYDTSKVASGVPARFSGSGSGTDYSLTINSLEAEDAATYYCQQWSSNPLTFGGGTKVEIK

SEQ ID NO: 15 - protein, 492 aa, Artificial sequence
DIVMTQSPSSLSVTPGERVSISCRSDKSLLHSNGNTYLYWFLQKPGQSPQVLIYRMSNLASGVPDRFSGSGSGTDFTLTISRVEAEDVGVYYCFQQLEYPYTFGQGTKLEIKGGGGSGGGGSGGGGSEVQLVQSGAELVKPGASVKLSCAASGFNIKDTYIYWVRQAPGQGLEWVGRIEPMNGNTKYDPKFQGRFTMTANTSKNTAYLQLSSLRSEDTAVYYCSRGGWLLLYVMDYWGQGTLVTVSSGGGGSDVQLVQSGAEVKKPGASVKVSCKASGYTFTRYTMHWVRQAPGQGLEWIGYINPSRGYTNYADSVKGRFTITTDKSTSTAYMELSSLRSEDTATYYCARYYDDHYCLDYWGQGTTVTVSSGGGGSGGGGSGGGGSDIVLTQSPATLSLSPGERATLSCRASQSVSYMNWYQQKPGKAPKRWIYDTSKVASGVPARFSGSGSGTDYSLTINSLEAEDAATYYCQQWSSNPLTFGGGTKVEIK

SEQ ID NO: 16 - protein, 246 aa, Artificial sequence
DIVLTQSPASLAVSLGQRATISCRASESVEYYGTSLMQWYQQKPGQPPKLLIYTASNVESGVPVRFSGSGSGTDFSLNIHPVEEDDIAMYFCQQSRKVPYTFGGGTKLEIKGGGGSGGGGSGGGGSQVQLQQSGPELMKPGASVKISCKATGYSFSGFWIEWVKQRPGHGLEWIGEILPGSGASNYHENFKGRATITADTSANTAYMQLRSLTSEDSAVYYCARERYYGSKYFDVWGAGTTVTVSS

SEQ ID NO: 17 - protein, 251 aa, Artificial sequence
DIVMTQAAPSVPVTPGESVSISCRSSKSLLHSNGNTYLYWFLQRPGQSPQLLISQMSNLASGIPDRFSGSGSGTAFTLRISRVEAEDVGVYYCMQHLEYPFTFGSGTKLEIKGGGGSGGGGSGGGGSEVQLQQSGAELVKPGASVKLSCTASGFNIKDNYMNWVKQRPEQGLEWIGRIDPANGNPKYDPKFQGKATITADTSSNTAYLQLSSLTSEDTAVYYCTRWIYYYGSRYEWYFDVWGAGTTVTVSS

SEQ ID NO: 18 - protein, 247 aa, Artificial sequence
DIVMTQAAPSVSVTPGESVSISCRSDKSLLHSNGNTYLYWFLQRPGQSPQVLIYRMSNLASGVPDRFSGSGSGTGFTLRVSRVEAEDVGVYYCFQQLEYPYTFGGGTKLEIKGGGGSGGGGSGGGGSEVQLQQSGAELVKPGASVKLSCTASGFNIKDTYIYWVKQRPGQGLEWIGRIEPMNGNTKYDPKFQGKATMTANTSSNTAYLHLSSLASEDTAVYFCSRGGWLLLYVMDYWGQGTSVTVSS

SEQ ID NO: 19 - protein, 242 aa, Artificial sequence
DIQMTQSPASLSASVGESVTITCRASENIYSYLTWYQQKQGKSPQLLVYNAKTLTEDVPSRFSGSGSGTQFSLKINSLQPEDFGSYYCQHHYGSPRTFGGGTKLEIKGGGGSGGGGSGGGGSQAQLQQSGAELMKPGASVKISCKATGYTFSNFWIEWVVQRPGHGLEWIGEILPGRGTTNYNEKFRGKATFTADTSSDTAYIQLSSLTSEDSAVYYCARERFYGSKYFDVWGAGTTVTVSS

SEQ ID NO: 20 - protein, 491 aa, Artificial sequence
DIVLTQSPASLAVSLGQRATISCRASESVEYYGTSLMQWYQQKPGQPPKLLIYTASNVESGVPVRFSGSGSGTDFSLNIHPVEEDDIAMYFCQQSRKVPYTFGGGTKLEIKGGGGSGGGGSGGGGSQVQLQQSGPELMKPGASVKISCKATGYSFSGFWIEWVKQRPGHGLEWIGEILPGSGASNYHENFKGRATITADTSANTAYMQLRSLTSEDSAVYYCARERYYGSKYFDVWGAGTTVTVSSGGGGSDVQLVQSGAEVKKPGASVKVSCKASGYTFTRYTMHWVRQAPGQGLEWIGYINPSRGYTNYADSVKGRFTITTDKSTSTAYMELSSLRSEDTATYYCARYYDDHYCLDYWGQGTTVTVSSGGGGSGGGGSGGGGSDIVLTQSPATLSLSPGERATLSCRASQSVSYMNWYQQKPGKAPKRWIYDTSKVASGVPARFSGSGSGTDYSLTINSLEAEDAATYYCQQWSSNPLTFGGGTKVEIK

SEQ ID NO: 21 - protein, 496 aa, Artificial sequence
DIVMTQAAPSVPVTPGESVSISCRSSKSLLHSNGNTYLYWFLQRPGQSPQLLISQMSNLASGIPDRFSGSGSGTAFTLRISRVEAEDVGVYYCMQHLEYPFTFGSGTKLEIKGGGGSGGGGSGGGGSEVQLQQSGAELVKPGASVKLSCTASGFNIKDNYMNWVKQRPEQGLEWIGRIDPANGNPKYDPKFQGKATITADTSSNTAYLQLSSLTSEDTAVYYCTRWIYYYGSRYEWYFDVWGAGTTVTVSSGGGGSDVQLVQSGAEVKKPGASVKVSCKASGYTFTRYTMHWVRQAPGQGLEWIGYINPSRGYTNYADSVKGRFTITTDKSTSTAYMELSSLRSEDTATYYCARYYDDHYCLDYWGQGTTVTVSSGGGGSGGGGSGGGGSDIVLTQSPATLSLSPGERATLSCRASQSVSYMNWYQQKPGKAPKRWIYDTSKVASGVPARFSGSGSGTDYSLTINSLEAEDAATYYCQQWSSNPLTFGGGTKVEIK

SEQ ID NO: 22 - protein, 492 aa, Artificial sequence
DIVMTQAAPSVSVTPGESVSISCRSDKSLLHSNGNTYLYWFLQRPGQSPQVLIYRMSNLASGVPDRFSGSGSGTGFTLRVSRVEAEDVGVYYCFQQLEYPYTFGGGTKLEIKGGGGSGGGGSGGGGSEVQLQQSGAELVKPGASVKLSCTASGFNIKDTYIYWVKQRPGQGLEWIGRIEPMNGNTKYDPKFQGKATMTANTSSNTAYLHLSSLASEDTAVYFCSRGGWLLLYVMDYWGQGTSVTVSSGGGGSDVQLVQSGAEVKKPGASVKVSCKASGYTFTRYTMHWVRQAPGQGLEWIGYINPSRGYTNYADSVKGRFTITTDKSTSTAYMELSSLRSEDTATYYCARYYDDHYCLDYWGQGTTVTVSSGGGGSGGGGSGGGGSDIVLTQSPATLSLSPGERATLSCRASQSVSYMNWYQQKPGKAPKRWIYDTSKVASGVPARFSGSGSGTDYSLTINSLEAEDAATYYCQQWSSNPLTFGGGTKVEIK

SEQ ID NO: 23 - protein, 487 aa, Artificial sequence
DIQMTQSPASLSASVGESVTITCRASENIYSYLTWYQQKQGKSPQLLVYNAKTLTEDVPSRFSGSGSGTQFSLKINSLQPEDFGSYYCQHHYGSPRTFGGGTKLEIKGGGGSGGGGSGGGGSQAQLQQSGAELMKPGASVKISCKATGYTFSNFWIEWVVQRPGHGLEWIGEILPGRGTTNYNEKFRGKATFTADTSSDTAYIQLSSLTSEDSAVYYCARERFYGSKYFDVWGAGTTVTVSSGGGGSDVQLVQSGAEVKKPGASVKVSCKASGYTFTRYTMHWVRQAPGQGLEWIGYINPSRGYTNYADSVKGRFTITTDKSTSTAYMELSSLRSEDTATYYCARYYDDHYCLDYWGQGTTVTVSSGGGGSGGGGSGGGGSDIVLTQSPATLSLSPGERATLSCRASQSVSYMNWYQQKPGKAPKRWIYDTSKVASGVPARFSGSGSGTDYSLTINSLEAEDAATYYCQQWSSNPLTFGGGTKVEIK

SEQ ID NO: 24 - protein, 20 aa, Artificial sequence
METDTLLLWVLLLWVPGSTG

SEQ ID NO: 25 - DNA, 798 bp, Artificial sequence
  source 1..798: mol_type = genomic DNA
atggagaccgacacactgctgctgtgggtgctgctgctgtgggtgccaggatccaccggcgacatcgtgctgacacagtcccctgctagcctggctgtgagcctgggccagagagccacaatctcttgccgcgctagcgagtctgtggagtactatggcaccagcctgatgcagtggtatcagcagaagcctggccagccccctaagctgctgatctacacagcctctaacgtggagtccggcgtgccagtgagattctccggcagcggctctggcaccgacttttccctgaatatccaccccgtggaggaggacgacatcgccatgtacttctgccagcagagccgcaaggtgccttatacctttggcggcggcacaaagctggagatcaagggcggcggcggctctggaggaggaggatccggaggaggaggaagccaggtgcagctgcagcagtctggaccagagctgatgaagccaggagctagcgtgaagatctcttgtaaggctaccggctattccttcagcggcttttggatcgagtgggtgaagcagaggccaggacacggactggagtggatcggagagatcctgccaggatctggagcttccaactatcatgagaatttcaagggcagggccaccatcacagctgacaccagcgccaacacagcttacatgcagctgcggagcctgacatctgaggattccgccgtgtactattgcgctagggagcggtactatggctctaagtactttgacgtgtggggagctggaaccacagtgaccgtgtccagc

SEQ ID NO: 26 - DNA, 813 bp, Artificial sequence
  source 1..813: mol_type = genomic DNA
atggagaccgacacactgctgctgtgggtgctgctgctgtgggtgcctggctctaccggcgacatcgtgatgacacaggctgctccatccgtgcctgtgacaccaggcgagagcgtgtctatctcctgcagatccagcaagtctctgctgcactccaacggcaatacctatctgtactggttcctgcagaggccaggacagagccctcagctgctgatctctcagatgtccaacctggcctctggcatccccgaccggttcagcggatctggatccggcaccgcctttacactgaggatcagccgggtggaggctgaggatgtgggcgtgtactattgcatgcagcatctggagtaccctttcacctttggctctggcacaaagctggagatcaagggaggaggaggatccggaggaggaggaagcggtggcggcggctctgaggtgcagctgcagcagtccggagctgagctggtgaagccaggagctagcgtgaagctgtcttgtaccgcctccggcttcaacatcaaggacaactacatgaattgggtgaagcagagaccagagcagggactggagtggatcggaaggatcgaccctgctaacggcaatccaaagtacgatcccaagtttcagggcaaggccaccatcacagctgacacctcttccaatacagcctatctgcagctgagctctctgacctccgaggatacagccgtgtactattgcacaagatggatctactattacggcagccgctatgagtggtactttgacgtgtggggagctggaaccacagtgaccgtgtccagc

SEQ ID NO: 27 - DNA, 801 bp, Artificial sequence
  source 1..801: mol_type = genomic DNA
atggagaccgacacactgctgctgtgggtgctgctgctgtgggtgccaggaagcaccggcgacatcgtgatgacacaggctgctccatccgtgtccgtgacaccaggcgagagcgtgtctatctcctgccgctctgataagtccctgctgcacagcaacggcaatacctacctgtattggttcctgcagagacccggccagtctcctcaggtgctgatctaccgcatgtctaacctggcctccggcgtgccagataggttcagcggatctggatccggaaccggctttacactgagggtgtctcgggtggaggctgaggacgtgggcgtgtactattgcttccagcagctggagtacccctatacctttggcggcggcacaaagctggagatcaagggaggaggaggatccggaggaggaggaagcggtggcggcggctctgaggtgcagctgcagcagtccggagctgagctggtgaagccaggagctagcgtgaagctgtcttgtaccgcctccggctttaatatcaaggatacatacatctattgggtgaagcagaggcctggacagggactggagtggatcggaaggatcgagcccatgaacggcaataccaagtacgaccctaagttccagggcaaggccaccatgacagctaacacctccagcaatacagcttatctgcatctgtcttccctggcctctgaggacaccgccgtgtacttttgctcccgcggaggatggctgctgctgtacgtgatggattattggggccagggcaccagcgtgacagtgagctct

SEQ ID NO: 28 - DNA, 786 bp, Artificial sequence
  source 1..786: mol_type = genomic DNA
atggagaccgacacactgctgctgtgggtgctgctgctgtgggtgccaggaagcaccggcgacatccagatgacacagtctccagcttctctgtccgctagcgtgggagagtccgtgaccatcacatgcagagctagcgagaacatctactcttatctgacctggtatcagcagaagcagggcaagtctccacagctgctggtgtacaatgccaagaccctgacagaggatgtgccatccaggttctctggatccggaagcggaacccagttttccctgaagatcaacagcctgcagcctgaggacttcggctcctactattgccagcaccattacggaagcccacggacctttggcggaggaacaaagctggagatcaagggcggcggcggctctggaggaggaggatccggaggaggaggaagccaggcccagctgcagcagagcggcgctgagctgatgaagccaggcgcctccgtgaagatcagctgtaaggctaccggctacacattctctaatttttggatcgagtgggtggtgcagaggcctggacacggactggagtggatcggagagatcctgccaggaaggggaaccacaaactataatgagaagttccggggcaaggccacctttacagctgacacctccagcgatacagcctacatccagctgtcttccctgacatccgaggacagcgccgtgtactattgcgctagggagcggttctacggctctaagtattttgacgtgtggggcgctggcaccacagtgaccgtgagctct

SEQ ID NO: 29 - DNA, 720 bp, Artificial sequence
  source 1..720: mol_type = genomic DNA
gatgtgcagctggtgcagagcggagctgaggtgaagaagccaggagcttctgtgaaggtgtcctgcaaagccagcggctacaccttcacaagatataccatgcactgggtgcgccaggctcctggacagggcctggaatggatcggctatatcaatccaagcagaggctacaccaactatgccgactctgtgaagggccgctttacaatcaccaccgataagtccaccagcacagcttacatggagctgagctctctgaggtccgaggacaccgccacatactattgcgctcggtactatgacgatcattactgtctggattattggggtcagggtaccacagtgaccgtgtcctctggcggcggcggcagcggcggaggaggctccggtggcggcggctccgacatcgtgctgacccagtcccctgccacactgtctctgtccccaggagagagagccaccctgagctgcagggctagccagtccgtgtcctacatgaattggtaccagcagaagccaggcaaggctcccaagaggtggatctatgatacatctaaggtggcctccggagtgcctgctcggttcagcggatctggatccggaaccgactacagcctgacaatcaattctctggaggccgaggatgccgctacctactattgtcagcagtggtcttccaacccactgacctttggcggcggcacaaaggtggagatcaag

SEQ ID NO: 30 - DNA, 15 bp, Artificial sequence
  source 1..15: mol_type = genomic DNA
ggaggaggaggatcc

SEQ ID NO: 31 - protein, 120 aa, Artificial sequence
EVQLQQSGAELVKPGASVKLSCTASGFNIKDTYIYWVKQRPGQGLEWIGRIEPMNGNTKYDPKFQGKATMTANTSSNTAYLHLSSLASEDTAVYFCSRGGWLLLYVMDYWGQGTSVTVSS

SEQ ID NO: 32 - protein, 113 aa, Artificial sequence
DIVMTQAAPSVSVTPGESVSISCRSDKSLLHSNGNTYLYWFLQRPGQSPQVLIYRMSNLASGVPDRFSGSGSGTGFTLRVSRVEAEDVGVYYCFQQLEYPYTFGGGTKLEIKR

SEQ ID NO: 33 - protein, 117 aa, Artificial sequence
EVQLQEAGPSLVKPSQTLSLTCFVTGDSITSGYWHWIRKFPGNKLEYMGYINYSGYTYYNPSLKSRFSITRDTSKNQYYLQLNSVTTEDTATYYCTSERNWGAFAYWGQGTLITVSS

SEQ ID NO: 34 - protein, 108 aa, Artificial sequence
ENVLTQSPAIMSASPGEKVTMTCRASSSVISTYLHWYQQKSGASPKLWIYSTSNLASGVPARFSGSGSGTSYSLTISSVEAEDAATYYCQQFSGYPYTFGGGTKLEIK

SEQ ID NO: 35 - protein, 112 aa, Artificial sequence
DIVMTQSASSLPVTPGESVSISCRSDKSLLHSNGNTYLYWFLQRPGQSPQVLIYRMSNLASGVPDRFSGSGSGTEFTLTISRVEAEDVGVYYCFQQLEYPYTFGPGTKLEIK

SEQ ID NO: 36 - protein, 120 aa, Artificial sequence
QVQLLQSGAEVVKPGASVKISCKASGFNIKDTYIYWVKQPTGQGLEWIGRIEPMNGNTKYDPKFQGRFTMTANTSINTAYLQLSSLTSEDTAVYYCSRGGWLLLYVMDYWGQGTTVTVSS

SEQ ID NO: 37 - protein, 112 aa, Artificial sequence
DIVMTQSPLSLSVTPGEPASISCRSDKSLLHSNGNTYLYWFLQKPGQSPQVLIYRMSNLASGVPDRFSGSGSGTDFTLKISRVEAEDVGVYYCFQQLEYPYTFGQGTKLEIK

SEQ ID NO: 38 - protein, 120 aa, Artificial sequence
QVQLVQSGAELVKPGASVKLSCKASGFNIKDTYIYWVRQAPGQGLEWIGRIEPMNGNTKYDPKFQGRVTMTANTSINTAYLELSSLRSEDTAVYYCSRGGWLLLYVMDYWGQGTLVTVSS

SEQ ID NO: 39 - protein, 108 aa, Artificial sequence
ENVLTQSPATLSVSPGEPVTLNCRASSSVISTYLHWYQQKPGQAPRLWIYSTSNLASGIPARFSGSGSGTEYTLTISSVESEDVAVYYCQQFSGYPYTFGQGTKLEIK

SEQ ID NO: 40 - protein, 117 aa, Artificial sequence
QVQLQESGPELVKPSQTLSLTCKVSGDSITSGYWHWIRQFPGRKLEWVGYINYSGYTYYNPSLKSRLTISRDTSKNQYFLELRSVTSDDTAVYYCTSERNWGAFAYWGQGTLITVSS

SEQ ID NO: 41 - protein, 108 aa, Artificial sequence
ENVLTQSPASLSVSPGERVTLNCRASSSVISTYLHWYQQKPGKPPRLWIYSTSNLASGIPARFSGSGSGTEYTLTISSVESEDFAVYYCQQFSGYPYTFGQGTKLEIK

SEQ ID NO: 42 - protein, 117 aa, Artificial sequence
QVQLQESGPELVKPSETLSLTCKVSGDSITSGYWHWIRQFPGQKLEYMGYINYSGYTYYNPSLKSRLTISRDTSKNQYFLKLRSVTSDDTALYYCTSERNWGAFAYWGQGTLITVSS

SEQ ID NO: 43 - protein, 108 aa, Artificial sequence
ENVLTQSPATLSASPGERATLSCRASSSVISTYLHWYQQKPGQAPKLWIYSTSNLASGVPARFSGSGSGTDYTLTISSVEPEDFAVYYCQQFSGYPYTFGQGTKLEIK

SEQ ID NO: 44 - protein, 117 aa, Artificial sequence
QVQLQESGPGLVKPSETLSLTCTVSGDSITSGYWHWIRQPPGKGLEWIGYINYSGYTYYNPSLKSRFTISRDTSKNQYYLQLNSVTAEDTAVYYCTSERNWGAFAYWGQGTLVTVSS

SEQ ID NO: 45 - protein, 108 aa, Artificial sequence
ENVLTQSPASLSASPGERVTITCRASSSVISTYLHWYQQKPGQAPKLWIYSTSNLASGVPARFSGSGSGTDYTLTISSVEPEDFATYYCQQFSGYPYTFGQGTKLEIK

SEQ ID NO: 46 - protein, 117 aa, Artificial sequence
EVQLQESGPGLVKPSGTLSLTCAVSGDSITSGYWHWIRQAPGKGLEWVGYINYSGYTYYNPSLKSRFTISRDTSKNQYYLQLNSVTAEDTAVYYCTSERNWGAFAYWGQGTLVTVSS

SEQ ID NO: 47 - protein, 107 aa, Artificial sequence
DILLTQSPSSLSATPGERATITCRASQGIRNNLNWYQQKPGQAPRLLIYYSSNLQSGVPSRFSGSGSGTDFTLTISRLQPEDVAAYYCQQSIKLPFTFGSGTKVEIK

SEQ ID NO: 48 - protein, 116 aa, Artificial sequence
EVQLVESGAGVKQPGGTLRLTCTASGFSLTTYGVHWVRQAPGKGLEWVGVIWGDGRTDYDAAFMSRVTISKDTSKSTVYLQMNSLRAEDTAVYYCMRNRHDWFDYWGQGTTVTVSS

SEQ ID NO: 49 - DNA, 816 bp, Artificial sequence
  source 1..816: mol_type = genomic DNA
atggagaccgacacactgctgctgtgggtgctgctgctgtgggtgccaggatccaccggcgacatcgtgatgacacagagcgcctccagcctgccagtgacccctggagagccagcttccatcagctgcagatctgacaagtccctgctgcacagcaacggcaatacatacctgtattggttcctgcagaagcccggccagtctcctcaggtgctgatctacagaatgagcaacctggcctctggagtgcctgaccgcttctctggatccggaagcggaaccgacttcaccctgacaatctctcgcgtggaggctgaggatgtgggcgtgtactattgcttccagcagctggagtacccatatacctttggccagggcacaaagctggagatcaagggaggaggaggatccggaggaggaggatctggcggcggcggctctcaggtgcagctggtgcagtccggagctgaggtggtgaagccaggagcttccgtgaagatcagctgtaaggcctctggcttcaatatcaaggacacctacatctattgggtgaggcagaggacaggacagggactggagtggatcggcaggatcgagccaatgaacggcaataccaagtacgatcccaagtttcagggccggctgaccatgacagccaacacctccaagaatacagcttatctgcagctgtcttccctgacctctgaggacacagccgtgtactattgttccaggggcggctggctgctgctgtacgtgatggattattggggccagggcaccacagtgacagtgagctctggcggcggcggcagc

SEQ ID NO: 50 - DNA, 819 bp, Artificial sequence
  source 1..819: mol_type = genomic DNA
atggagcacagcaccttcctgtctggcctggtgctggccacactgctgtcccaggtgagccctgacatcgtgatgacccagtccgcttccagcctgcctgtgacacctggagagtccgtgagcatctcttgccggtctgataagtccctgctgcatagcaacggcaatacctacctgtattggtttctgcagaggccaggccagtctccccaggtgctgatctacaggatgtccaacctggccagcggagtgccagacagattctccggcagcggctctggcacagagtttaccctgacaatctctagagtggaggctgaggatgtgggcgtgtactattgcttccagcagctggagtacccttatacctttggcccaggcacaaagctggagatcaagggcggcggcggctctggaggaggaggatccggaggaggaggcagccaggtgcagctgctgcagtccggagctgaggtggtgaagccaggagcttctgtgaagatctcctgtaaggccagcggcttcaatatcaaggacacctacatctattgggtgaagcagccaacaggacagggcctggagtggatcggaaggatcgagcccatgaacggcaataccaagtacgatcctaagttccagggcaggtttaccatgacagccaacacctccatcaatacagcttatctgcagctgtcttccctgacctctgaggacacagccgtgtactattgttcccgcggaggatggctgctgctgtacgtgatggattattggggccagggcaccacagtgaccgtgagctctggcggcggcggcagc

SEQ ID NO: 51 - DNA, 819 bp, Artificial sequence
  source 1..819: mol_type = genomic DNA
atggagcactccaccttcctgagcggcctggtgctggccacactgctgtctcaggtgtcccctgacatcgtgatgacccagtccccactgagcctgtctgtgacacccggcgagcctgcttccatcagctgcagaagcgataagtctctgctgcattccaacggcaatacctacctgtattggtttctgcagaagccaggccagagcccccaggtgctgatctacaggatgtctaacctggcctccggagtgcctgaccggttctctggatccggaagcggaaccgacttcaccctgaagatctccagggtggaggctgaggacgtgggcgtgtactattgcttccagcagctggagtacccatatacctttggccagggcacaaagctggagatcaagggaggaggaggaagcggaggaggaggatctggcggcggcggctcccaggtgcagctggtgcagtctggagctgagctggtgaagccaggagctagcgtgaagctgtcttgtaaggcctccggcttcaatatcaaggacacctacatctattgggtgaggcaggctccaggacagggcctggagtggatcggaaggatcgagcccatgaacggcaatacaaagtacgatcctaagtttcagggcagggtgaccatgacagccaacacctctatcaatacagcttatctggagctgtccagcctgagaagcgaggacaccgccgtgtactattgttctcgcggcggctggctgctgctgtacgtgatggattattggggccagggcaccctggtgacagtgtcttccggaggaggaggatcc

SEQ ID NO: 52 - DNA, 819 bp, Artificial sequence
  source 1..819: mol_type = genomic DNA
atggagcactccaccttcctgagcggcctggtgctggccacactgctgtctcaggtgtcccccgacatcgtgatgacccagagcccatccagcctgtctgtgacaccaggagagagggtgtccatcagctgccggagcgataagtctctgctgcattctaacggcaatacctacctgtattggtttctgcagaagcccggccagtcccctcaggtgctgatctacagaatgtctaacctggcctccggagtgccagaccgcttctctggatccggaagcggcacagacttcaccctgacaatctccagggtggaggctgaggacgtgggcgtgtactattgcttccagcagctggagtacccctatacctttggccagggcacaaagctggagatcaagggaggaggaggatccggaggaggaggaagcggcggcggcggctctgaggtgcagctggtgcagtccggagctgagctggtgaagccaggagctagcgtgaagctgtcttgtgccgcttccggcttcaatatcaaggacacctacatctattgggtgagacaggctcctggacagggcctggagtgggtgggccgcatcgagcctatgaacggcaatacaaagtacgatccaaagttccagggcaggtttaccatgacagccaacaccagcaagaatacagcttatctgcagctgtcttccctgaggtccgaggacaccgccgtgtactattgtagccggggaggatggctgctgctgtacgtgatggattattggggccagggcaccctggtgacagtgagctctggaggaggaggatct

SEQ ID NO: 53 - DNA, 795 bp, Artificial sequence
  source 1..795: mol_type = genomic DNA
atggagaccgacacactgctgctgtgggtgctgctgctgtgggtgccaggaagcaccggagagaacgtgctgacccagtctcctgccacactgagcgtgtctcccggcgagcctgtgaccctgaattgcagggcttccagctctgtgatcagcacatatctgcactggtaccagcagaagccaggacaggctcccaggctgtggatctattccaccagcaacctggcctctggcatccctgctcggttctctggatccggaagcggcacagagtacaccctgacaatctccagcgtggagtccgaggatgtggccgtgtactattgccagcagttcagcggctacccatatacctttggccagggcacaaagctggagatcaagggaggaggaggaagcggaggaggaggatctggcggcggcggctcccaggtgcagctgcaggagtccggacctgagctggtgaagccatcccagaccctgagcctgacctgtaaggtgtctggcgactccatcaccagcggctactggcattggatcaggcagtttccaggccggaagctggagtgggtgggctacatcaactatagcggctacacatactataatccctctctgaagtccagactgaccatctccagggacacatccaagaaccagtatttcctggagctgagaagcgtgacctctgacgatacagccgtgtactattgtacctctgagcgcaattggggcgcctttgcttactggggccagggcaccctgatcacagtgtctagcggcggcggcggctcc

SEQ ID NO: 54 - DNA, 816 bp, Artificial sequence
  source 1..816: mol_type = genomic DNA
atggagcactccaccttcctgagcggcctggtgctggccacactgctgtcccaggtgagccctgagaacgtgctgacccagtctcctgctagcctgtccgtgtccccaggagagagagtgaccctgaattgccgcgcttccagctctgtgatctccacatacctgcattggtatcagcagaagccaggcaagccacccaggctgtggatctacagcacctctaacctggcctctggcatccctgctcggttctccggaagcggatctggcacagagtacaccctgacaatctccagcgtggagtccgaggactttgccgtgtactattgccagcagttcagcggctacccatatacctttggccagggcacaaagctggagatcaagggaggaggaggatccggaggaggaggaagcggcggcggcggctctcaggtgcagctgcaggagtccggcccagagctggtgaagccctctgagacactgtccctgacctgtaaggtgtctggcgactccatcaccagcggctactggcactggatcaggcagtttccaggccagaagctggagtacatgggctatatcaactacagcggctatacatactataatccctctctgaagtccaggctgaccatcagccgggatacatctaagaaccagtacttcctgaagctgagaagcgtgacctctgacgatacagccctgtactattgtaccagcgagcgcaattggggcgcctttgcttattggggccagggcaccctgatcacagtgtcttccggcggcggcggctctgatgtgcagctggtgcag

SEQ ID NO: 55 - DNA, 816 bp, Artificial sequence
  source 1..816: mol_type = genomic DNA
atggagcactccaccttcctgagcggcctggtgctggccacactgctgtctcaggtgtcccctgagaacgtgctgacccagtctccagccacactgtccgcctctcctggagagagagccaccctgtcctgcagggcttccagctctgtgatcagcacatatctgcattggtaccagcagaagccaggccaggcccccaagctgtggatctattccaccagcaatctggccagcggcgtgccagctaggttctctggctccggcagcggcacagactacaccctgacaatctccagcgtggagccagaggattttgccgtgtactattgccagcagttctctggctacccctatacctttggccagggcacaaagctggagatcaagggaggaggaggatccggaggaggaggaagcggcggcggcggctctcaggtgcagctgcaggagtccggacctggcctggtgaagccatctgagacactgtccctgacctgtacagtgagcggcgactctatcacatccggctattggcactggatcaggcagccacctggcaagggcctggagtggatcggctacatcaactatagcggctacacctactataatcccagcctgaagtctaggttcaccatcagccgggacacatctaagaaccagtactatctgcagctgaattctgtgaccgccgaggatacagccgtgtactattgtacctccgagagaaactggggcgcctttgcttactggggccagggcaccctggtgacagtgtcttccggaggaggaggatccgatgtgcagctggtgcag

SEQ ID NO: 56 - DNA, 798 bp, Artificial sequence
  source 1..798: mol_type = genomic DNA
atggagcacagcaccttcctgtctggcctggtgctggccacactgctgtcccaggtgagccctgagaacgtgctgacccagtcccctgctagcctgtctgcttccccaggagagagagtgaccatcacatgccgcgcctccagctctgtgatcagcacctatctgcattggtaccagcagaagcccggccaggctcctaagctgtggatctatagcacatctaatctggcctctggagtgccagctaggttctccggaagcggatctggaaccgactacaccctgacaatctccagcgtggagcccgaggattttgctacatactattgccagcagttctccggctacccttatacctttggccagggcacaaagctggagatcaagggaggaggaggaagcggaggaggaggatctggcggcggcggctccgaggtgcagctgcaggagagcggaccaggcctggtgaagccatccggcaccctgagcctgacatgtgccgtgtctggcgactccatcaccagcggctattggcactggatcaggcaggctccaggcaagggcctggagtgggtgggctacatcaactattctggctacacatactataatccctctctgaagtccaggttcaccatctctcgggacacatccaagaaccagtactatctgcagctgaatagcgtgaccgccgaggatacagccgtgtactattgtacctctgagagaaactggggcgcctttgcttactggggccagggcaccctggtgacagtgtcttccggaggaggaggatcc

SEQ ID NO: 57 - protein, 246 aa, Artificial sequence
QVQLVQSGAEVKKPGSSVKVSCKASGFAFTDYYIHWVRQAPGQGLEWMGWISPGNVNTKYNENFKGRVTITADKSTSTAYMELSSLRSEDTAVYYCARDGYSLYYFDYWGQGTLVTVSSGGGGSGGGGSGGGGSDIVMTQSPDSLAVSLGERATINCKSSQSLLNSRTRKNYLAWYQQKPGQPPKLLIYWASTRQSGVPDRFSGSGSGTDFTLTISSLQAEDVAVYYCTQSHTLRTFGGGTKVEIK